European Patent Specification EP 3 286 326 B1, published January 22, 2025. Title: METHODS AND COMPOSITIONS FOR WHOLE TRANSCRIPTOME AMPLIFICATION. Applicant: Cellular Research, Inc. Fu, Glenn Betts, Craig Fan, Christina Lam, Gretchen Yinbon. The sequence listing filed with the application follows.

SEQUENCE LISTING (38 sequences)

SEQ ID NO: 1 - DNA, 30 bp, Artificial Sequence
  CBO102
gcgatcgcgatcggaagagcacacgtctga

SEQ ID NO: 2 - DNA, 17 bp, Artificial Sequence
  CBO103
cttccgatcgcgatcgc

SEQ ID NO: 3 - DNA, 18 bp, Artificial Sequence
  CBO23
tcagacgtgtgctcttcc

SEQ ID NO: 4 - DNA, 26 bp, Artificial Sequence
  CBO105
gcgatcgcggaagagcacacgtctga

SEQ ID NO: 5 - DNA, 16 bp, Artificial Sequence
  CBO106
gctcttccgcgatcgc

SEQ ID NO: 6 - DNA, 18 bp, Artificial Sequence
  CBO23
tcagacgtgtgctcttcc

SEQ ID NO: 7 - DNA, 21 bp, Artificial Sequence
  CBO17
tcagacgtgtgctcttccgat

SEQ ID NO: 8 - DNA, 26 bp, Artificial Sequence
  CBO105
gcgatcgcggaagagcacacgtctga

SEQ ID NO: 9 - DNA, 17 bp, Artificial Sequence
  CBO107
gctcttccgcgatcgct

SEQ ID NO: 10 - DNA, 18 bp, Artificial Sequence
  CBO23
tcagacgtgtgctcttcc

SEQ ID NO: 11 - DNA, 55 bp, Artificial Sequence
  CBO16
tcagacgtgtgctcttccgatctgcgatcgctttttttttttttttttttttttt

SEQ ID NO: 12 - DNA, 30 bp, Artificial Sequence
  CBO12
  misc_feature (25)...(30): n = random nucleotide
ccctacacgacgctcttccgatctnnnnnn

SEQ ID NO: 13 - DNA, 70 bp, Artificial Sequence
  CBO32
aatgatacggcgaccaccgagatctacactatagcctacactctttccctacacgacgctcttccgatct

SEQ ID NO: 14 - DNA, 66 bp, Artificial Sequence
  CBO33
caagcagaagacggcatacgagatcgagtaatgtgactggagttcagacgtgtgctcttccgatct

SEQ ID NO: 15 - DNA, 53 bp, Artificial Sequence
  CBO10
tcagacgtgtgctcttccgatgcgatcgctttttttttttttttttttttttt

SEQ ID NO: 16 - DNA, 24 bp, Artificial Sequence
  Illumina Read 1
ccctacacgacgctcttccgatct

SEQ ID NO: 17 - DNA, 17 bp, Artificial Sequence
  CBO122
cttccgatcgcgatcgc

SEQ ID NO: 18 - DNA, 29 bp, Artificial Sequence
  CBO103
gcgatcgcgatcggaagagcgtcgtgtag

SEQ ID NO: 19 - DNA, 16 bp, Artificial Sequence
  CBO123
gctcttccgcgatcgc

SEQ ID NO: 20 - DNA, 25 bp, Artificial Sequence
  CBO106
gcgatcgcggaagagcgtcgtgtag

SEQ ID NO: 21 - DNA, 14 bp, Artificial Sequence
  Poly-A
aaaaaaaaaaaaaa

SEQ ID NO: 22 - DNA, 14 bp, Artificial Sequence
  Oligo dT
tttttttttttttt

SEQ ID NO: 23 - DNA, 14 bp, Artificial Sequence
  Poly-A
aaaaaaaaaaaaaa

SEQ ID NO: 24 - DNA, 14 bp, Artificial Sequence
  Oligo dT
tttttttttttttt

SEQ ID NO: 25 - DNA, 13 bp, Artificial Sequence
  Poly-A
aaaaaaaaaaaaa

SEQ ID NO: 26 - DNA, 14 bp, Artificial Sequence
  Oligo dT
tttttttttttttt

SEQ ID NO: 27 - DNA, 18 bp, Artificial Sequence
  Universal sequence 1
cttccgctagcgatcgct

SEQ ID NO: 28 - DNA, 30 bp, Artificial Sequence
  Universal sequence 2
agcgatcgcgatcggaagagcgtcgtgtag

SEQ ID NO: 29 - DNA, 18 bp, Artificial Sequence
  CBO40
ctacacgacgctcttccg

SEQ ID NO: 30 - DNA, 20 bp, Artificial Sequence
  ILR2
acacgacgctcttccgatct

SEQ ID NO: 31 - DNA, 34 bp, Artificial Sequence
  Transposome sequence P7
ctgtctcttatacacatctccgagcccacgagac

SEQ ID NO: 32 - DNA, 22 bp, Artificial Sequence
  Universal sequence 3
ctacacgacgctcttccgatct

SEQ ID NO: 33 - DNA, 19 bp, Artificial Sequence
  Transposase primer
agatgtgtataagagacag

SEQ ID NO: 34 - DNA, 33 bp, Artificial Sequence
  Transposome sequence P5
ctgtctcttatacacatctgacgctgccgacga

SEQ ID NO: 35 - DNA, 62 bp, Artificial Sequence
  P5
aatgatacggcgaccaccgagatctacacacactctttccctacacgacgctcttccgatct

SEQ ID NO: 36 - DNA, 19 bp, Artificial Sequence
  Transposome sequence
ctgtctcttatacacatct

SEQ ID NO: 37 - DNA, 58 bp, Artificial Sequence
  P7
caagcagaagacggcatacgagatgtctcgtgggctcggagatgtgtataagagacag

SEQ ID NO: 38 - DNA, 20 bp, Artificial Sequence
  Universal sequence 4
acacgacgctcttccgatct